European Patent Application EP 4 807 009 A1, published September 16, 2026. Title: 一种重组表达猫血清白蛋白的方法. Applicant: 北京舜雷科技有限公司. Application CN. The sequence listing filed with the application follows.

SEQUENCE LISTING (18 sequences)

SEQ ID NO: 1 - protein, 584 aa, synthetic construct
EAHQSEIAHRFNDLGEEHFRGLVLVAFSQYLQQCPFEDHVKLVNEVTEFAKGCVADQSAANCEKSLHELLGDKLCTVASLRDKYGEMADCCEKKEPERNECFLQHKDDNPGFGQLVTPEADAMCTAFHENEQRFLGKYLYEIARRHPYFYAPELLYYAEEYKGVFTECCEAADKAACLTPKVDALREKVLASSAKERLKCASLQKFGERAFKAWSVARLSQKFPKAEFAEISKLVTDLAKIHKECCHGDLLECADDRADLAKYICENQDSISTKLKECCGKPVLEKSHCISEVERDELPADLPPLAVDFVEDKEVCKNYQEAKDVFLGTFLYEYSRRHPEYSVSLLLRLAKEYEATLEKCCATDDPPACYAHVFDEFKPLVEEPHNLVKTNCELFEKLGEYGFQNALLVRYTKKVPQVSTPTLVEVSRSLGKVGSKCCTHPEAERLSCAEDYLSVVLNRLCVLHEKTPVSERVTKCCTESLVNRRPCFSALQVDETYVPKEFSAETFTFHADLCTLPEAEKQIKKQSALVELLKHKPKATEEQLKTVMGDFGSFVDKCCAAEDKEACFAEEGPKLVAAAQAALA

SEQ ID NO: 2 - DNA, 1755 bp, synthetic construct
  source 1..1755: mol_type = other DNA
gaagctcatcaatctgaaattgctcatagatttaacgatttgggtgaagaacattttagaggtttggttttggttgctttctctcaatacttgcaacaatgtccattcgaagaccacgttaagttggttaacgaagttactgaattcgctaagggttgtgttgctgaccaatctgctgctaactgtgaaaagtctttgcacgaattgttgggtgacaagttgtgtactgttgcttctttgagagacaagtacggtgaaatggctgactgttgtgaaaagaaggaaccagaaagaaacgaatgtttcttgcaacacaaggacgacaacccaggtttcggtcaattggttactccagaagctgacgctatgtgtactgctttccacgaaaacgaacaaagattcttgggtaagtacttgtacgaaatcgctagaagacacccatacttctacgctccagaattgttgtactacgctgaagaatacaagggtgttttcactgaatgttgtgaagctgctgacaaggctgcttgtttgactccaaaggttgacgctttgagagaaaaggttttggcttcttctgctaaggaaagattgaagtgtgcttctttgcaaaagttcggtgaaagagctttcaaggcttggtctgttgctagattgtctcaaaagttcccaaaggctgaattcgctgaaatctctaagttggttactgacttggctaagatccacaaggaatgttgtcacggtgacttgttggaatgtgctgacgacagagctgacttggctaagtacatctgtgaaaaccaagactctatctctactaagttgaaggaatgttgtggtaagccagttttggaaaagtctcactgtatctctgaagttgaaagagacgaattgccagctgacttgccaccattggctgttgacttcgttgaagacaaggaagtttgtaagaactaccaagaagctaaggacgttttcttgggtactttcttgtacgaatactctagaagacacccagaatactctgtttctttgttgttgagattggctaaggaatacgaagctactttggaaaagtgttgtgctactgacgacccaccagcttgttacgctcacgttttcgacgaattcaagccattggttgaagaaccacacaacttggttaagactaactgtgaattgttcgaaaagttgggtgaatacggtttccaaaacgctttgttggttagatacactaagaaggttccacaagtttctactccaactttggttgaagtttctagatctttgggtaaggttggttctaagtgttgtactcacccagaagctgaaagattgtcttgtgctgaagactacttgtctgttgttttgaacagattgtgtgttttgcacgaaaagactccagtttctgaaagagttactaagtgttgtactgaatctttggttaacagaagaccatgtttctctgctttgcaagttgacgaaacttacgttccaaaggaattctctgctgaaactttcactttccacgctgacttgtgtactttgccagaagctgaaaagcaaatcaagaagcaatctgctttggttgaattgttgaagcacaagccaaaggctactgaagaacaattgaagactgttatgggtgacttcggttctttcgttgacaagtgttgtgctgctgaagacaaggaagcttgtttcgctgaagaaggtccaaagttggttgctgctgctcaagctgctttggcttaa

SEQ ID NO: 3 - DNA, 43 bp, synthetic construct
  source 1..43: mol_type = other DNA
gaagaaggggtatctctcgagaaaagagaagctcatcaatctg

SEQ ID NO: 4 - DNA, 36 bp, synthetic construct
  source 1..36: mol_type = other DNA
ataagaatgcggccgcttaagccaaagcagcttgag

SEQ ID NO: 5 - protein, 495 aa, synthetic construct
SDQEAIAPEDSHVVKLTEATFESFITSNPHVLAEFFAPWCGHCKKLGPELVSAAEILKDNEQVKIAQIDCTEEKELCQGYEIKGYPTLKVFHGEVEVPSDYQGQRQSQSIVSYMLKQSLPPVSEINATKDLDDTIAEAKEPVIVQVLPEDASNLESNTTFYGVAGTLREKFTFVSTKSTDYAKKYTSDSTPAYLLVRPGEEPSVYSGEELDETHLVHWIDIESKPLFGDIDGSTFKSYAEANIPLAYYFYENEEQRAAAADIIKPFAKEQRGKINFVGLDAVKFGKHAKNLNMDEEKLPLFVIHDLVSNKKFGVPQDQELTNKDVTELIEKFIAGEAEPIVKSEPIPEIQEEKVFKLVGKAHDEVVFDESKDVLVKYYAPWCGHCKRMAPAYEELATLYANDEDASSKVVIAKLDHTLNDVDNVDIQGYPTLILYPAGDKSNPQLYDGSRDLESLAEFVKERGTHKVDALALRPVEEEKEAEEEAESEADAHDEL

SEQ ID NO: 6 - DNA, 1488 bp, synthetic construct
  source 1..1488: mol_type = other DNA
tctgaccaagaagctatcgctccagaagactctcacgttgttaagttgactgaagctactttcgaatctttcatcacttctaacccacacgttttggctgaattcttcgctccatggtgtggtcactgtaagaagttgggtccagaattggtttctgctgctgaaatcttgaaggacaacgaacaagttaagatcgctcaaatcgactgtactgaagaaaaggaattgtgtcaaggttacgaaatcaagggttacccaactttgaaggttttccacggtgaagttgaagttccatctgactaccaaggtcaaagacaatctcaatctatcgtttcttacatgttgaagcaatctttgccaccagtttctgaaatcaacgctactaaggacttggacgacactatcgctgaagctaaggaaccagttatcgttcaagttttgccagaagacgcttctaacttggaatctaacactactttctacggtgttgctggtactttgagagaaaagttcactttcgtttctactaagtctactgactacgctaagaagtacacttctgactctactccagcttacttgttggttagaccaggtgaagaaccatctgtttactctggtgaagaattggacgaaactcacttggttcactggatcgacatcgaatctaagccattgttcggtgacatcgacggttctactttcaagtcttacgctgaagctaacatcccattggcttactacttctacgaaaacgaagaacaaagagctgctgctgctgacatcatcaagccattcgctaaggaacaaagaggtaagatcaacttcgttggtttggacgctgttaagttcggtaagcacgctaagaacttgaacatggacgaagaaaagttgccattgttcgttatccacgacttggtttctaacaagaagttcggtgttccacaagaccaagaattgactaacaaggacgttactgaattgatcgaaaagttcatcgctggtgaagctgaaccaatcgttaagtctgaaccaatcccagaaatccaagaagaaaaggttttcaagttggttggtaaggctcacgacgaagttgttttcgacgaatctaaggacgttttggttaagtactacgctccatggtgtggtcactgtaagagaatggctccagcttacgaagaattggctactttgtacgctaacgacgaagacgcttcttctaaggttgttatcgctaagttggaccacactttgaacgacgttgacaacgttgacatccaaggttacccaactttgatcttgtacccagctggtgacaagtctaacccacaattgtacgacggttctagagacttggaatctttggctgaattcgttaaggaaagaggtactcacaaggttgacgctttggctttgagaccagttgaagaagaaaaggaagctgaagaagaagctgaatctgaagctgacgctcacgacgaattgtaa

SEQ ID NO: 7 - DNA, 44 bp, synthetic construct
  source 1..44: mol_type = other DNA
gaagaaggggtatctctcgagaaaagatctgaccaagaagctat

SEQ ID NO: 8 - DNA, 40 bp, synthetic construct
  source 1..40: mol_type = other DNA
gttctagaaagctggcggccgcttacaattcgtcgtgagc

SEQ ID NO: 9 - protein, 330 aa, synthetic construct
MPVDSSHKIASPLPPRKRAKTEEEKEQRRVERILRNRRAAHASREKKRRHVEFLENHVVDLESALQESAKATNKLKQIQDIIVSRLEALGGTVSDLDLAVPEVDFPKFSDLELSTDLSSSTKSEKASTSTCRSSTEDLDEDGVAEYDDEEDEELPRKKNVLNDKSKNRTIKQEKLNELPSPLSSDFSDVDEEKSTLTHFQLQQQQQQQPVDNYVSTPLSLPEDSIDFINPGSLKIESDENFLLGSSTLQIKHENDTEYIPTAPSGSINDFFNSYDISESNRLHHPAVMTDSSLHTTAGSIGFFSLIRGKSFVVGRRSSVGVYQLTCIAIR

SEQ ID NO: 10 - DNA, 993 bp, synthetic construct
  source 1..993: mol_type = other DNA
atgccagttgactcttctcacaagatcgcttctccattgccaccaagaaagagagctaagactgaagaagaaaaggaacaaagaagagttgaaagaatcttgagaaacagaagagctgctcacgcttctagagaaaagaagagaagacacgttgaattcttggaaaaccacgttgttgacttggaatctgctttgcaagaatctgctaaggctactaacaagttgaagcaaatccaagacatcatcgtttctagattggaagctttgggtggtactgtttctgacttggacttggctgttccagaagttgacttcccaaagttctctgacttggaattgtctactgacttgtcttcttctactaagtctgaaaaggcttctacttctacttgtagatcttctactgaagacttggacgaagacggtgttgctgaatacgacgacgaagaagacgaagaattgccaagaaagaagaacgttttgaacgacaagtctaagaacagaactatcaagcaagaaaagttgaacgaattgccatctccattgtcttctgacttctctgacgttgacgaagaaaagtctactttgactcacttccaattgcaacaacaacaacaacaacaaccagttgacaactacgtttctactccattgtctttgccagaagactctatcgacttcatcaacccaggttctttgaagatcgaatctgacgaaaacttcttgttgggttcttctactttgcaaatcaagcacgaaaacgacactgaatacatcccaactgctccatctggttctatcaacgacttcttcaactcttacgacatctctgaatctaacagattgcaccacccagctgttatgactgactcttctttgcacactactgctggttctatcggtttcttctctttgatcagaggtaagtctttcgttgttggtagaagatcttctgttggtgtttaccaattgacttgtatcgctatcagataa

SEQ ID NO: 11 - DNA, 36 bp, synthetic construct
  source 1..36: mol_type = other DNA
caactaattattcgaaacgatgccagttgactcttc

SEQ ID NO: 12 - DNA, 42 bp, synthetic construct
  source 1..42: mol_type = other DNA
gttctagaaagctggcggccgcttatctgatagcgatacaag

SEQ ID NO: 13 - protein, 146 aa, synthetic construct
MLDQQTINIIKATVPVLKEHGVTITTTFYKNLFAKHPEVRPLFDMGRQESLEQPKALAMTVLAAAQNIENLPAILPAVKKIAVKHCQAGVAAAHYPIVGQELLGAIKEVLGDAATDDILDAWGKAYGVIADVFIQVEADLYAQAVE

SEQ ID NO: 14 - DNA, 441 bp, synthetic construct
  source 1..441: mol_type = other DNA
atgttggaccaacaaactatcaacatcatcaaggctactgttccagttttgaaggaacacggtgttactatcactactactttctacaagaacttgttcgctaagcacccagaagttagaccattgttcgacatgggtagacaagaatctttggaacaaccaaaggctttggctatgactgttttggctgctgctcaaaacatcgaaaacttgccagctatcttgccagctgttaagaagatcgctgttaagcactgtcaagctggtgttgctgctgctcactacccaatcgttggtcaagaattgttgggtgctatcaaggaagttttgggtgacgctgctactgacgacatcttggacgcttggggtaaggcttacggtgttatcgctgacgttttcatccaagttgaagctgacttgtacgctcaagctgttgaataa

SEQ ID NO: 15 - DNA, 37 bp, synthetic construct
  source 1..37: mol_type = other DNA
caactaattattcgaaacgatgttggaccaacaaact

SEQ ID NO: 16 - DNA, 41 bp, synthetic construct
  source 1..41: mol_type = other DNA
gttctagaaagctggcggccgcttattcaacagcttgagcg

SEQ ID NO: 17 - DNA, 65 bp, synthetic construct
  source 1..65: mol_type = other DNA
cttgtatcgctatcagataagcggccgccaactaattattcgaaacgatgttggaccaacaaact

SEQ ID NO: 18 - DNA, 38 bp, synthetic construct
  source 1..38: mol_type = other DNA
cgctcaagctgttgaataatctagaacaaaaactcatc